European Patent Specification EP 3 344 291 B1, published November 27, 2024. Title: VACCINE COMPOSITIONS HAVING IMPROVED STABILITY AND IMMUNOGENICITY. Applicant: Novavax, Inc. Smith, Gale Liu, Ye Tian, Jing-Hui Massare, Michael J. Boddapati, Sarathi Shane, Erica Oliver, Cynthia. The sequence listing filed with the application follows.

SEQUENCE LISTING (29 sequences)

SEQ ID NO: 1 - DNA, 1725 bp, Respiratory syncytial virus
atggagttgctaatcctcaaagcaaatgcaattaccacaatcctcactgcagtcacattttgttttgcttctggtcaaaacatcactgaagaattttatcaatcaacatgcagtgcagttagcaaaggctatcttagtgctctgagaactggttggtataccagtgttataactatagaattaagtaatatcaaggaaaataagtgtaatggaacagatgctaaggtaaaattgataaaacaagaattagataaatataaaaatgctgtaacagaattgcagttgctcatgcaaagcacaccaccaacaaacaatcgagccagaagagaactaccaaggtttatgaattatacactcaacaatgccaaaaaaaccaatgtaacattaagcaagaaaaggaaaagaagatttcttggttttttgttaggtgttggatctgcaatcgccagtggcgttgctgtatctaaggtcctgcacctagaaggggaagtgaacaagatcaaaagtgctctactatccacaaacaaggctgtagtcagcttatcaaatggagttagtgtcttaaccagcaaagtgttagacctcaaaaactatatagataaacaattgttacctattgtgaacaagcaaagctgcagcatatcaaatatagaaactgtgatagagttccaacaaaagaacaacagactactagagattaccagggaatttagtgttaatgcaggtgtaactacacctgtaagcacttacatgttaactaatagtgaattattgtcattaatcaatgatatgcctataacaaatgatcagaaaaagttaatgtccaacaatgttcaaatagttagacagcaaagttactctatcatgtccataataaaagaggaagtcttagcatatgtagtacaattaccactatatggtgttatagatacaccctgttggaaactacacacatcccctctatgtacaaccaacacaaaagaagggtccaacatctgtttaacaagaactgacagaggatggtactgtgacaatgcaggatcagtatctttcttcccacaagctgaaacatgtaaagttcaatcaaatcgagtattttgtgacacaatgaacagtttaacattaccaagtgaaataaatctctgcaatgttgacatattcaaccccaaatatgattgtaaaattatgacttcaaaaacagatgtaagcagctccgttatcacatctctaggagccattgtgtcatgctatggcaaaactaaatgtacagcatccaataaaaatcgtggaatcataaagacattttctaacgggtgcgattatgtatcaaataaagggatggacactgtgtctgtaggtaacacattatattatgtaaataagcaagaaggtaaaagtctctatgtaaaaggtgaaccaataataaatttctatgacccattagtattcccctctgatgaatttgatgcatcaatatctcaagtcaacgagaagattaaccagagcctagcatttattcgtaaatccgatgaattattacataatgtaaatgctggtaaatccaccacaaatatcatgataactactataattatagtgattatagtaatattgttatcattaattgctgttggactgctcttatactgtaaggccagaagcacaccagtcacactaagcaaagatcaactgagtggtataaataatattgcatttagtaactaa

SEQ ID NO: 2 - protein, 574 aa, Respiratory syncytial virus
MELLILKANAITTILTAVTFCFASGQNITEEFYQSTCSAVSKGYLSALRTGWYTSVITIELSNIKENKCNGTDAKVKLIKQELDKYKNAVTELQLLMQSTPPTNNRARRELPRFMNYTLNNAKKTNVTLSKKRKRRFLGFLLGVGSAIASGVAVSKVLHLEGEVNKIKSALLSTNKAVVSLSNGVSVLTSKVLDLKNYIDKQLLPIVNKQSCSISNIETVIEFQQKNNRLLEITREFSVNAGVTTPVSTYMLTNSELLSLINDMPITNDQKKLMSNNVQIVRQQSYSIMSIIKEEVLAYVVQLPLYGVIDTPCWKLHTSPLCTTNTKEGSNICLTRTDRGWYCDNAGSVSFFPQAETCKVQSNRVFCDTMNSLTLPSEINLCNVDIFNPKYDCKIMTSKTDVSSSVITSLGAIVSCYGKTKCTASNKNRGIIKTFSNGCDYVSNKGMDTVSVGNTLYYVNKQEGKSLYVKGEPIINFYDPLVFPSDEFDASISQVNEKINQSLAFIRKSDELLHNVNAGKSTTNIMITTIIIVIIVILLSLIAVGLLLYCKARSTPVTLSKDQLSGINNIAFSN

SEQ ID NO: 3 - protein, 573 aa, Artificial Sequence
  Deletion of 137 (delta 1)
MELLILKANAITTILTAVTFCFASGQNITEEFYQSTCSAVSKGYLSALRTGWYTSVITIELSNIKENKCNGTDAKVKLIKQELDKYKNAVTELQLLMQSTPATNNRARRELPRFMNYTLNNAKKTNVTLSKKQKQQLGFLLGVGSAIASGVAVSKVLHLEGEVNKIKSALLSTNKAVVSLSNGVSVLTSKVLDLKNYIDKQLLPIVNKQSCSISNIETVIEFQQKNNRLLEITREFSVNAGVTTPVSTYMLTNSELLSLINDMPITNDQKKLMSNNVQIVRQQSYSIMSIIKEEVLAYVVQLPLYGVIDTPCWKLHTSPLCTTNTKEGSNICLTRTDRGWYCDNAGSVSFFPQAETCKVQSNRVFCDTMNSLTLPSEVNLCNVDIFNPKYDCKIMTSKTDVSSSVITSLGAIVSCYGKTKCTASNKNRGIIKTFSNGCDYVSNKGVDTVSVGNTLYYVNKQEGKSLYVKGEPIINFYDPLVFPSDEFDASISQVNEKINQSLAFIRKSDELLHNVNAGKSTTNIMITTIIIVIIVILLSLIAVGLLLYCKARSTPVTLSKDQLSGINNIAFSN

SEQ ID NO: 4 - protein, 572 aa, Artificial Sequence
  Deletion of 137-138 (delta 2)
MELLILKANAITTILTAVTFCFASGQNITEEFYQSTCSAVSKGYLSALRTGWYTSVITIELSNIKENKCNGTDAKVKLIKQELDKYKNAVTELQLLMQSTPATNNRARRELPRFMNYTLNNAKKTNVTLSKKQKQQGFLLGVGSAIASGVAVSKVLHLEGEVNKIKSALLSTNKAVVSLSNGVSVLTSKVLDLKNYIDKQLLPIVNKQSCSISNIETVIEFQQKNNRLLEITREFSVNAGVTTPVSTYMLTNSELLSLINDMPITNDQKKLMSNNVQIVRQQSYSIMSIIKEEVLAYVVQLPLYGVIDTPCWKLHTSPLCTTNTKEGSNICLTRTDRGWYCDNAGSVSFFPQAETCKVQSNRVFCDTMNSLTLPSEVNLCNVDIFNPKYDCKIMTSKTDVSSSVITSLGAIVSCYGKTKCTASNKNRGIIKTFSNGCDYVSNKGVDTVSVGNTLYYVNKQEGKSLYVKGEPIINFYDPLVFPSDEFDASISQVNEKINQSLAFIRKSDELLHNVNAGKSTTNIMITTIIIVIIVILLSLIAVGLLLYCKARSTPVTLSKDQLSGINNIAFSN

SEQ ID NO: 5 - protein, 571 aa, Artificial Sequence
  Deletion of 137-139 (delta 3)
MELLILKANAITTILTAVTFCFASGQNITEEFYQSTCSAVSKGYLSALRTGWYTSVITIELSNIKENKCNGTDAKVKLIKQELDKYKNAVTELQLLMQSTPATNNRARRELPRFMNYTLNNAKKTNVTLSKKQKQQFLLGVGSAIASGVAVSKVLHLEGEVNKIKSALLSTNKAVVSLSNGVSVLTSKVLDLKNYIDKQLLPIVNKQSCSISNIETVIEFQQKNNRLLEITREFSVNAGVTTPVSTYMLTNSELLSLINDMPITNDQKKLMSNNVQIVRQQSYSIMSIIKEEVLAYVVQLPLYGVIDTPCWKLHTSPLCTTNTKEGSNICLTRTDRGWYCDNAGSVSFFPQAETCKVQSNRVFCDTMNSLTLPSEVNLCNVDIFNPKYDCKIMTSKTDVSSSVITSLGAIVSCYGKTKCTASNKNRGIIKTFSNGCDYVSNKGVDTVSVGNTLYYVNKQEGKSLYVKGEPIINFYDPLVFPSDEFDASISQVNEKINQSLAFIRKSDELLHNVNAGKSTTNIMITTIIIVIIVILLSLIAVGLLLYCKARSTPVTLSKDQLSGINNIAFSN

SEQ ID NO: 6 - protein, 570 aa, Artificial Sequence
  Deletion of 137-140 (delta 4)
MELLILKANAITTILTAVTFCFASGQNITEEFYQSTCSAVSKGYLSALRTGWYTSVITIELSNIKENKCNGTDAKVKLIKQELDKYKNAVTELQLLMQSTPATNNRARRELPRFMNYTLNNAKKTNVTLSKKQKQQLLGVGSAIASGVAVSKVLHLEGEVNKIKSALLSTNKAVVSLSNGVSVLTSKVLDLKNYIDKQLLPIVNKQSCSISNIETVIEFQQKNNRLLEITREFSVNAGVTTPVSTYMLTNSELLSLINDMPITNDQKKLMSNNVQIVRQQSYSIMSIIKEEVLAYVVQLPLYGVIDTPCWKLHTSPLCTTNTKEGSNICLTRTDRGWYCDNAGSVSFFPQAETCKVQSNRVFCDTMNSLTLPSEVNLCNVDIFNPKYDCKIMTSKTDVSSSVITSLGAIVSCYGKTKCTASNKNRGIIKTFSNGCDYVSNKGVDTVSVGNTLYYVNKQEGKSLYVKGEPIINFYDPLVFPSDEFDASISQVNEKINQSLAFIRKSDELLHNVNAGKSTTNIMITTIIIVIIVILLSLIAVGLLLYCKARSTPVTLSKDQLSGINNIAFSN

SEQ ID NO: 7 - protein, 569 aa, Artificial Sequence
  Deletion of 137-141 (delta 5)
MELLILKANAITTILTAVTFCFASGQNITEEFYQSTCSAVSKGYLSALRTGWYTSVITIELSNIKENKCNGTDAKVKLIKQELDKYKNAVTELQLLMQSTPATNNRARRELPRFMNYTLNNAKKTNVTLSKKQKQQLGVGSAIASGVAVSKVLHLEGEVNKIKSALLSTNKAVVSLSNGVSVLTSKVLDLKNYIDKQLLPIVNKQSCSISNIETVIEFQQKNNRLLEITREFSVNAGVTTPVSTYMLTNSELLSLINDMPITNDQKKLMSNNVQIVRQQSYSIMSIIKEEVLAYVVQLPLYGVIDTPCWKLHTSPLCTTNTKEGSNICLTRTDRGWYCDNAGSVSFFPQAETCKVQSNRVFCDTMNSLTLPSEVNLCNVDIFNPKYDCKIMTSKTDVSSSVITSLGAIVSCYGKTKCTASNKNRGIIKTFSNGCDYVSNKGVDTVSVGNTLYYVNKQEGKSLYVKGEPIINFYDPLVFPSDEFDASISQVNEKINQSLAFIRKSDELLHNVNAGKSTTNIMITTIIIVIIVILLSLIAVGLLLYCKARSTPVTLSKDQLSGINNIAFSN

SEQ ID NO: 8 - protein, 564 aa, Artificial Sequence
  Deletion of 137-146 (delta 10)
MELLILKANAITTILTAVTFCFASGQNITEEFYQSTCSAVSKGYLSALRTGWYTSVITIELSNIKENKCNGTDAKVKLIKQELDKYKNAVTELQLLMQSTPATNNRARRELPRFMNYTLNNAKKTNVTLSKKQKQQAIASGVAVSKVLHLEGEVNKIKSALLSTNKAVVSLSNGVSVLTSKVLDLKNYIDKQLLPIVNKQSCSISNIETVIEFQQKNNRLLEITREFSVNAGVTTPVSTYMLTNSELLSLINDMPITNDQKKLMSNNVQIVRQQSYSIMSIIKEEVLAYVVQLPLYGVIDTPCWKLHTSPLCTTNTKEGSNICLTRTDRGWYCDNAGSVSFFPQAETCKVQSNRVFCDTMNSLTLPSEVNLCNVDIFNPKYDCKIMTSKTDVSSSVITSLGAIVSCYGKTKCTASNKNRGIIKTFSNGCDYVSNKGVDTVSVGNTLYYVNKQEGKSLYVKGEPIINFYDPLVFPSDEFDASISQVNEKINQSLAFIRKSDELLHNVNAGKSTTNIMITTIIIVIIVILLSLIAVGLLLYCKARSTPVTLSKDQLSGINNIAFSN

SEQ ID NO: 9 - protein, 568 aa, Artificial Sequence
  Deletion of 137-142 (delta 6)
MELLILKANAITTILTAVTFCFASGQNITEEFYQSTCSAVSKGYLSALRTGWYTSVITIELSNIKENKCNGTDAKVKLIKQELDKYKNAVTELQLLMQSTPATNNRARRELPRFMNYTLNNAKKTNVTLSKKQKQQGVGSAIASGVAVSKVLHLEGEVNKIKSALLSTNKAVVSLSNGVSVLTSKVLDLKNYIDKQLLPIVNKQSCSISNIETVIEFQQKNNRLLEITREFSVNAGVTTPVSTYMLTNSELLSLINDMPITNDQKKLMSNNVQIVRQQSYSIMSIIKEEVLAYVVQLPLYGVIDTPCWKLHTSPLCTTNTKEGSNICLTRTDRGWYCDNAGSVSFFPQAETCKVQSNRVFCDTMNSLTLPSEVNLCNVDIFNPKYDCKIMTSKTDVSSSVITSLGAIVSCYGKTKCTASNKNRGIIKTFSNGCDYVSNKGVDTVSVGNTLYYVNKQEGKSLYVKGEPIINFYDPLVFPSDEFDASISQVNEKINQSLAFIRKSDELLHNVNAGKSTTNIMITTIIIVIIVILLSLIAVGLLLYCKARSTPVTLSKDQLSGINNIAFSN

SEQ ID NO: 10 - protein, 567 aa, Artificial Sequence
  Deletion of 137-143 (delta 7)
MELLILKANAITTILTAVTFCFASGQNITEEFYQSTCSAVSKGYLSALRTGWYTSVITIELSNIKENKCNGTDAKVKLIKQELDKYKNAVTELQLLMQSTPATNNRARRELPRFMNYTLNNAKKTNVTLSKKQKQQVGSAIASGVAVSKVLHLEGEVNKIKSALLSTNKAVVSLSNGVSVLTSKVLDLKNYIDKQLLPIVNKQSCSISNIETVIEFQQKNNRLLEITREFSVNAGVTTPVSTYMLTNSELLSLINDMPITNDQKKLMSNNVQIVRQQSYSIMSIIKEEVLAYVVQLPLYGVIDTPCWKLHTSPLCTTNTKEGSNICLTRTDRGWYCDNAGSVSFFPQAETCKVQSNRVFCDTMNSLTLPSEVNLCNVDIFNPKYDCKIMTSKTDVSSSVITSLGAIVSCYGKTKCTASNKNRGIIKTFSNGCDYVSNKGVDTVSVGNTLYYVNKQEGKSLYVKGEPIINFYDPLVFPSDEFDASISQVNEKINQSLAFIRKSDELLHNVNAGKSTTNIMITTIIIVIIVILLSLIAVGLLLYCKARSTPVTLSKDQLSGINNIAFSN

SEQ ID NO: 11 - protein, 566 aa, Artificial Sequence
  Deletion of 137-144 (delta 8)
MELLILKANAITTILTAVTFCFASGQNITEEFYQSTCSAVSKGYLSALRTGWYTSVITIELSNIKENKCNGTDAKVKLIKQELDKYKNAVTELQLLMQSTPATNNRARRELPRFMNYTLNNAKKTNVTLSKKQKQQGSAIASGVAVSKVLHLEGEVNKIKSALLSTNKAVVSLSNGVSVLTSKVLDLKNYIDKQLLPIVNKQSCSISNIETVIEFQQKNNRLLEITREFSVNAGVTTPVSTYMLTNSELLSLINDMPITNDQKKLMSNNVQIVRQQSYSIMSIIKEEVLAYVVQLPLYGVIDTPCWKLHTSPLCTTNTKEGSNICLTRTDRGWYCDNAGSVSFFPQAETCKVQSNRVFCDTMNSLTLPSEVNLCNVDIFNPKYDCKIMTSKTDVSSSVITSLGAIVSCYGKTKCTASNKNRGIIKTFSNGCDYVSNKGVDTVSVGNTLYYVNKQEGKSLYVKGEPIINFYDPLVFPSDEFDASISQVNEKINQSLAFIRKSDELLHNVNAGKSTTNIMITTIIIVIIVILLSLIAVGLLLYCKARSTPVTLSKDQLSGINNIAFSN

SEQ ID NO: 12 - protein, 565 aa, Artificial Sequence
  Deletion of 137-145 (delta 9)
MELLILKANAITTILTAVTFCFASGQNITEEFYQSTCSAVSKGYLSALRTGWYTSVITIELSNIKENKCNGTDAKVKLIKQELDKYKNAVTELQLLMQSTPATNNRARRELPRFMNYTLNNAKKTNVTLSKKQKQQSAIASGVAVSKVLHLEGEVNKIKSALLSTNKAVVSLSNGVSVLTSKVLDLKNYIDKQLLPIVNKQSCSISNIETVIEFQQKNNRLLEITREFSVNAGVTTPVSTYMLTNSELLSLINDMPITNDQKKLMSNNVQIVRQQSYSIMSIIKEEVLAYVVQLPLYGVIDTPCWKLHTSPLCTTNTKEGSNICLTRTDRGWYCDNAGSVSFFPQAETCKVQSNRVFCDTMNSLTLPSEVNLCNVDIFNPKYDCKIMTSKTDVSSSVITSLGAIVSCYGKTKCTASNKNRGIIKTFSNGCDYVSNKGVDTVSVGNTLYYVNKQEGKSLYVKGEPIINFYDPLVFPSDEFDASISQVNEKINQSLAFIRKSDELLHNVNAGKSTTNIMITTIIIVIIVILLSLIAVGLLLYCKARSTPVTLSKDQLSGINNIAFSN

SEQ ID NO: 13 - protein, 565 aa, Artificial Sequence
  Deletion of 137-145 (delta 9) with wild type fusion cleavage site
MELLILKANAITTILTAVTFCFASGQNITEEFYQSTCSAVSKGYLSALRTGWYTSVITIELSNIKENKCNGTDAKVKLIKQELDKYKNAVTELQLLMQSTPATNNRARRELPRFMNYTLNNAKKTNVTLSKKRKRRSAIASGVAVSKVLHLEGEVNKIKSALLSTNKAVVSLSNGVSVLTSKVLDLKNYIDKQLLPIVNKQSCSISNIETVIEFQQKNNRLLEITREFSVNAGVTTPVSTYMLTNSELLSLINDMPITNDQKKLMSNNVQIVRQQSYSIMSIIKEEVLAYVVQLPLYGVIDTPCWKLHTSPLCTTNTKEGSNICLTRTDRGWYCDNAGSVSFFPQAETCKVQSNRVFCDTMNSLTLPSEVNLCNVDIFNPKYDCKIMTSKTDVSSSVITSLGAIVSCYGKTKCTASNKNRGIIKTFSNGCDYVSNKGVDTVSVGNTLYYVNKQEGKSLYVKGEPIINFYDPLVFPSDEFDASISQVNEKINQSLAFIRKSDELLHNVNAGKSTTNIMITTIIIVIIVILLSLIAVGLLLYCKARSTPVTLSKDQLSGINNIAFSN

SEQ ID NO: 14 - protein, 6 aa, Artificial Sequence
  mutated furin cleavage site
KKQKQQ

SEQ ID NO: 15 - protein, 6 aa, Artificial Sequence
  mutated furin cleavage site
QKQKQQ

SEQ ID NO: 16 - protein, 6 aa, Artificial Sequence
  mutated furin cleavage site
KKQKRQ

SEQ ID NO: 17 - protein, 6 aa, Artificial Sequence
  mutated furin cleavage site
GRRQQR

SEQ ID NO: 18 - protein, 6 aa, Unknown
  furin cleavage site
KKRKRR

SEQ ID NO: 19 - protein, 539 aa, Artificial Sequence
  modified RSV F protein
QNITEEFYQSTCSAVSKGYLSALRTGWYTSVITIELSNIKENKCNGTDAKVKLIKQELDKYKNAVTELQLLMQSTPATNNRARRELPRFMNYTLNNAKKTNVTLSKKQKQQAIASGVAVSKVLHLEGEVNKIKSALLSTNKAVVSLSNGVSVLTSKVLDLKNYIDKQLLPIVNKQSCSISNIETVIEFQQKNNRLLEITREFSVNAGVTTPVSTYMLTNSELLSLINDMPITNDQKKLMSNNVQIVRQQSYSIMSIIKEEVLAYVVQLPLYGVIDTPCWKLHTSPLCTTNTKEGSNICLTRTDRGWYCDNAGSVSFFPQAETCKVQSNRVFCDTMNSLTLPSEVNLCNVDIFNPKYDCKIMTSKTDVSSSVITSLGAIVSCYGKTKCTASNKNRGIIKTFSNGCDYVSNKGVDTVSVGNTLYYVNKQEGKSLYVKGEPIINFYDPLVFPSDEFDASISQVNEKINQSLAFIRKSDELLHNVNAGKSTTNIMITTIIIVIIVILLSLIAVGLLLYCKARSTPVTLSKDQLSGINNIAFSN

SEQ ID NO: 20 - protein, 19 aa, Artificial Sequence
  portions of antigenic site II
NSELLSLINDMPITNDQKK

SEQ ID NO: 21 - protein, 5 aa, Artificial Sequence
  portions of antigenic site II
LMSNN

SEQ ID NO: 22 - protein, 676 aa, Ebola virus
MGVTGILQLPRDRFKRTSFFLWVIILFQRTFSIPLGVIHNSTLQVSDVDKLVCRDKLSSTNQLRSVGLNLEGNGVATDVPSVTKRWGFRSGVPPKVVNYEAGEWAENCYNLEIKKPDGSECLPAAPDGIRGFPRCRYVHKVSGTGPCAGDFAFHKEGAFFLYDRLASTVIYRGTTFAEGVVAFLILPQAKKDFFSSHPLREPVNATEDPSSGYYSTTIRYQATGFGTNETEYLFEVDNLTYVQLESRFTPQFLLQLNETIYASGKRSNTTGKLIWKVNPEIDTTIGEWAFWETKKNLTRKIRSEELSFTAVSNGPKNISGQSPARTSSDPETNTTNEDHKIMASENSSAMVQVHSQGRKAAVSHLTTLATISTSPQPPTTKTGPDNSTHNTPVYKLDISEATQVGQHHRRADNDSTASDTPPATTAAGPLKAENTNTSKSADSLDLATTTSPQNYSETAGNNNTHHQDTGEESASSGKLGLITNTIAGVAGLITGGRRTRREVIVNAQPKCNPNLHYWTTQDEGAAIGLAWIPYFGPAAEGIYTEGLMHNQDGLICGLRQLANETTQALQLFLRATTELRTFSILNRKAIDFLLQRWGGTCHILGPDCCIEPHDWTKNITDKIDQIIHDFVDKTLPDQGDNDNWWTGWRQWIPAGIGVTGVIIAVIALFCICKFVF

SEQ ID NO: 23 - protein, 17 aa, Ebola virus
HNTPVYKLDISEATQVE

SEQ ID NO: 24 - protein, 17 aa, Ebola virus
ATQVEQHHRRTDNDSTA

SEQ ID NO: 25 - protein, 17 aa, Ebola virus
ATQVGQHHRRADNDSTA

SEQ ID NO: 26 - protein, 25 aa, Respiratory syncytial virus
MELLILKANAITTILTAVTFCFASG

SEQ ID NO: 27 - protein, 676 aa, Ebola virus
MGVTGILQLPRDRFKRTSFFLWVIILFQRTFSIPLGVIHNSTLQVSDVDKLVCRDKLSSTNQLRSVGLNLEGNGVATDVPSATKRWGFRSGVPPKVVNYEAGEWAENCYNLEIKKPDGSECLPAAPDGIRGFPRCRYVHKVSGTGPCAGDFAFHKEGAFFLYDRLASTVIYRGTTFAEGVVAFLILPQAKKDFFSSHPLREPVNATEDPSSGYYSTTIRYQATGFGTNETEYLFEVDNLTYVQLESRFTPQFLLQLNETIYTSGKRSNTTGKLIWKVNPEIDTTIGEWAFWETKKNLTRKIRSEELSFTVVSNGAKNISGQSPARTSSDPGTNTTTEDHKIMASENSSAMVQVHSQGREAAVSHLTTLATISTSPQSLTTKPGPDNSTHNTPVYKLDISEATQVEQHHRRTDNDSTASDTPSATTAAGPPKAENTNTSKSTDFLDPATTTSPQNHSETAGNNNTHHQDTGEESASSGKLGLITNTIAGVAGLITGGRRTRREAIVNAQPKCNPNLHYWTTQDEGAAIGLAWIPYFGPAAEGIYIEGLMHNQDGLICGLRQLANETTQALQLFLRATTELRTFSILNRKAIDFLLQRWGGTCHILGPDCCIEPHDWTKNITDKIDQIIHDFVDKTLPDQGDNDNWWTGWRQWIPAGIGVTGVIIAVIALFCICKFVF

SEQ ID NO: 28 - protein, 676 aa, Ebola virus; identical to SEQ ID NO: 22

SEQ ID NO: 29 - protein, 644 aa, Ebola virus
IPLGVIHNSTLQVSDVDKLVCRDKLSSTNQLRSVGLNLEGNGVATDVPSVTKRWGFRSGVPPKVVNYEAGEWAENCYNLEIKKPDGSECLPAAPDGIRGFPRCRYVHKVSGTGPCAGDFAFHKEGAFFLYDRLASTVIYRGTTFAEGVVAFLILPQAKKDFFSSHPLREPVNATEDPSSGYYSTTIRYQATGFGTNETEYLFEVDNLTYVQLESRFTPQFLLQLNETIYASGKRSNTTGKLIWKVNPEIDTTIGEWAFWETKKNLTRKIRSEELSFTAVSNGPKNISGQSPARTSSDPETNTTNEDHKIMASENSSAMVQVHSQGRKAAVSHLTTLATISTSPQPPTTKTGPDNSTHNTPVYKLDISEATQVGQHHRRADNDSTASDTPPATTAAGPLKAENTNTSKSADSLDLATTTSPQNYSETAGNNNTHHQDTGEESASSGKLGLITNTIAGVAGLITGGRRTRREVIVNAQPKCNPNLHYWTTQDEGAAIGLAWIPYFGPAAEGIYTEGLMHNQDGLICGLRQLANETTQALQLFLRATTELRTFSILNRKAIDFLLQRWGGTCHILGPDCCIEPHDWTKNITDKIDQIIHDFVDKTLPDQGDNDNWWTGWRQWIPAGIGVTGVIIAVIALFCICKFVF